European Patent Application EP 4 603 502 A1, published August 20, 2025. Title: Peptide Having Activity of Promoting Hair Growth and Inhibiting Hair Loss and Uses Thereof. Applicant: CAREGENE CO., LTD. Application KR. The sequence listing filed with the application follows.

SEQUENCE LISTING (15 sequences)

SEQ ID NO: 1 - protein, 8 aa, synthetic construct
LKRYKHLV

SEQ ID NO: 2 - DNA, 20 bp, synthetic construct
  source 1..20: mol_type = other DNA
ccagctattgtaacacctca

SEQ ID NO: 3 - DNA, 20 bp, synthetic construct
  source 1..20: mol_type = other DNA
ttcagatgtaggcagctgtc

SEQ ID NO: 4 - DNA, 25 bp, synthetic construct
  source 1..25: mol_type = other DNA
accagcagcgactctgaggaggaac

SEQ ID NO: 5 - DNA, 26 bp, synthetic construct
  source 1..26: mol_type = other DNA
tgaccctcttggcagcaggatagtcc

SEQ ID NO: 6 - DNA, 20 bp, synthetic construct
  source 1..20: mol_type = other DNA
ggagccaaaagggtcatcat

SEQ ID NO: 7 - DNA, 20 bp, synthetic construct
  source 1..20: mol_type = other DNA
gtgatggcatggactgtggt

SEQ ID NO: 8 - DNA, 20 bp, synthetic construct
  source 1..20: mol_type = other DNA
gatcatcgagctgagacgca

SEQ ID NO: 9 - DNA, 20 bp, synthetic construct
  source 1..20: mol_type = other DNA
ctggccccagggtatctagt

SEQ ID NO: 10 - DNA, 20 bp, synthetic construct
  source 1..20: mol_type = other DNA
ccctcaaggatgccaggaac

SEQ ID NO: 11 - DNA, 19 bp, synthetic construct
  source 1..19: mol_type = other DNA
cactgctacctccggcaag

SEQ ID NO: 12 - DNA, 20 bp, synthetic construct
  source 1..20: mol_type = other DNA
ccaaatccgcaccaaggtca

SEQ ID NO: 13 - DNA, 21 bp, synthetic construct
  source 1..21: mol_type = other DNA
gtattgattgccaggaggggg

SEQ ID NO: 14 - DNA, 20 bp, synthetic construct
  source 1..20: mol_type = other DNA
cgcggcgtatccgtgtcctc

SEQ ID NO: 15 - DNA, 24 bp, synthetic construct
  source 1..24: mol_type = other DNA
agcctgttccgtctcaaacttggt